European Patent Specification EP 3 119 186 B1, published September 20, 2023. Title: Transgenic Maize Event MON 87419 and Methods of Use Thereof. Applicant: Monsanto Technology LLC. Application Unknown. The sequence listing filed with the application follows.

SEQUENCE LISTING (22 sequences)

SEQ ID NO: 1 - DNA, 30 bp, Artificial Sequence
  Recombinant
caggtattgatgtgcgccagtcagcatcat

SEQ ID NO: 2 - DNA, 30 bp, Artificial Sequence
  Recombinant
ttctttttctccatagcattcgcaatacag

SEQ ID NO: 3 - DNA, 60 bp, Artificial Sequence
  Recombinant
gcaggcggtcgctgccaggtattgatgtgcgccagtcagcatcatcacaccaaaagttag

SEQ ID NO: 4 - DNA, 60 bp, Artificial Sequence
  Recombinant
attggtaattactctttctttttctccatagcattcgcaatacagttagatgcgagtgaa

SEQ ID NO: 5 - DNA, 100 bp, Artificial Sequence
  Recombinant
aggggggggttggcggggtggcaggcggtcgctgccaggtattgatgtgcgccagtcagcatcatcacaccaaaagttaggcccgaatagtttgaaatta

SEQ ID NO: 6 - DNA, 100 bp, Artificial Sequence
  Recombinant
catttttgaattgaaaaaaaattggtaattactctttctttttctccatagcattcgcaatacagttagatgcgagtgaagcacgataagtcacaaccat

SEQ ID NO: 7 - DNA, 1771 bp, Artificial Sequence
  Recombinant
gttgatattttgacccaaagacatgccattctcattgttttcagttttatcctaccaatgtagtaacccaaacagtttaattacaagtgaatcaactggaaacaagatctacagactgcacacagcacattaacaattctgcgccaaatgaatgacagagtgatttataggcactaagctggttttcatcatgaattttgatcagagcataaaccttgttgacaacagaatagaatcaaacaagctgctcagctcagatggaccaaaataatgaacgcgcgcacagtatattgaaccaaaatagtgaacgcacagtagaaaacagacggagaagctagtgcacactaaaaatagaactcactgatgcatttttaaccgaatcattaaaaaacagaccaacatgattagaccagctatcaaaagacacactgctgagaatcaacaactgctatatgtgtgatctacctgaaataaacagatgcagttttttgtccctacagaccaacatgttttaatcagaatgccaatgataaatccttagagatctggagagcaaactaattaaccactgagaatcaacaactgctataatccttagagatctggagagcacactaattaaccactgagcctctttggtcagcatgcagaaatccccaaaactatactgtaattcgaaacccataagcgcacatcaaagcaactccattgttgatggttgggaatgttaaaaatatggttgtggacaccaattgccgtaaacaaacccacagggagaacatgagtatgaacaatcaaaactaacatgaataagtggatgttcagattaagtaaggaaaatggtgcacagattaagaacagagcaatgtatagcacaagtggaaattacaaaccttttttcacaaaattacaatctctagacagcacacagcaagatcttggaatggatgagggtgatgaatcggtgaaaaaagacagcacacagcaagatctctagaacagaacatgaaatgttggagagtggggatgggttgtagacctaacctctgtccatccttttaatagccgtcgctgccaggtatggaatagggcgccgtgagtgccgtcgagggcgcgcgcaggggcgcggtttggtgtgggcgggatacccggcgcggtcgggaaaccccacggcggtcatcacggcgagccgggggaggggggggttggcggggtggcaggcggtcgctgccaggtattgatgtgcgccagtcagcatcatcacaccaaaagttaggcccgaatagtttgaaattagaaagctcgcaattgaggtctgtcgaggaggttaacctaggtactgaattaccctgttatccctaactagatatcgaattctaactataacggtcctaaggtagcgaatcgttcttcttggcgcgccaagacgcaaactcggaccggttcaagccgtcaaggcacttctatgcaaccacagtcaacttgaatgccgcttgagtgccttctcaagtttttttttcttgcaaaaatcatttcttttttttaaaaaaagtataatttggatcgtgcaaatttctctctaggtgtgtgtgtgactgtgtgagtaacaatttctctagttgtgcgcgactgctgcttactttggagattacaatatctttctaaaatgcttcgattacttatttataaaccgtctctaaggccaattgctcaagattcattcaacaattgaaacgtctcacatgattaaatcatataaagtttctaagtc

SEQ ID NO: 8 - DNA, 1767 bp, Artificial Sequence
  Recombinant
gcgagtctgatgagacatctctgtattgtgtttctttccccagtgttttctgtacttgtgtaatcggctaatcgccaacagattcggcgatgaataaatgagaaataaattgttctgattttgagtgcaaaaaaaaaggaattagatctgtgtgtgttttttggatccccggggcggccgcacaacaaacgaatacgtcctgcttggcctactaggccaacgcaggcgctggccgtgacggccacgagcgaactgatatcgaattctagggataacagggtaatccacgtgtagctaaacgcgccctcatctaagcccccatttggacgtgaatgtagacacgtcgaaataaagatttccgaattagaataatttgtttattgctttcgcctataaatacgacggatcgtaatttgtcgttttatcaaaatgtactttcattttataataacgctgcggacatctacatttttgaattgaaaaaaaattggtaattactctttctttttctccatagcattcgcaatacagttagatgcgagtgaagcacgataagtcacaaccataatacatactattagaatccggctctttgccgagtgctttttttgggcactcggcaaagacttctttaccggcaaagtcctactctcggtaacgaccacgtttaccgagagcaggacgctcggtacagggagacactcggcaaagacctctttgtcgagtgccaaacgctcggcaaagggccgtcagcagccgtctatagcagatgtttattatctttgccgagcgccaagcgttggcactcggcaaaacaagtgttgccgagtgcttaaattggacactcggcaaaatatatttttcttttttctttttgcaaccaaactttctgtggtttgttcctacactatgtagacatacatgttccattttggcacaattataaaagtgtttgctataaatattagattttgttcgtttaattgaattttctcggataattcagatttgaactacaagtcactcaaaaaatggaaaaccatgaatgcaaaaatgatatccatgttatttagcacaagttacggccgatttcaggagtagacccgaatttttgagcaccatgctcacgaaacatgactgtgaacttgtcatccagttgttttaaaattgtataaaacacaaacaaaatcaaaaaatcatgaaacttgtccacatgtcatgatatcatcatatgtagaggttgtgataaaaagttgaaaatatttcgtgaaagttgtccatagttcactgagcctctttgtcgagtgtcacactcggcaaagcctttgtcgagtgcttcagacactcggcaaataagttgtttccagtagtgacattaatagaaaaagagtgcatagttcgttcacatagctaactaattggttcattacaaagaaacattagaacaagcataatgatgacttggacataatgaaataaaatacataggttgagggaaccaaacataatggaacacagaacaaatagaggacaacatcatagaaaacgacataacttcacatgggttttacgccaattgctccacgccaagtccataagtgctcgatgagatcatgttgaagttggttgtatcatttgagactagtgatgttgtggtgggagcatagccactctgtacgaacttcagggattgtgatgagagatccacgtgcactccaattgcggcaaactcaacattacttgcacgtgggaccttgtcctcgacaa

SEQ ID NO: 9 - DNA, 6762 bp, Artificial Sequence
  Recombinant
gccagtcagcatcatcacaccaaaagttaggcccgaatagtttgaaattagaaagctcgcaattgaggtctgtcgaggaggttaacctaggtactgaattaccctgttatccctaactagatatcgaattctaactataacggtcctaaggtagcgaatcgttcttcttggcgcgccaagacgcaaactcggaccggttcaagccgtcaaggcacttctatgcaaccacagtcaacttgaatgccgcttgagtgccttctcaagtttttttttcttgcaaaaatcatttcttttttttaaaaaaagtataatttggatcgtgcaaatttctctctaggtgtgtgtgtgactgtgtgagtaacaatttctctagttgtgcgcgactgctgcttactttggagattacaatatctttctaaaatgcttcgattacttatttataaaccgtctctaaggccaattgctcaagattcattcaacaattgaaacgtctcacatgattaaatcatataaagtttctaagtcttgtttgacaagatttttttagattttcatctaaattggatgaaactatcaaacactaattttaaaaaatataagagaagctccggagataaaaggtcgtctatgttattataagagtaaagtcgtctattctcttcgtcccaacatatataattctaagcatgaattgctttctttttggacaaaaggagcatgccacaacacaagaatgatgtcaccgtcatgcttggatccttttatggtaaagcttcaccttctataatctaacaatagagaaatcagggaaaaatcatgttttggttgtttttatttctaacctccacaataactttggtttaccattttttgtttgattttagttttagagaagcgtttataacaggacctaaaatcttttttcagtacacagtacaacgcagacgctcatacacgcacgcacactcacctctatgaacacacgtaagaaaaccctacaccttgagcaccttcgaaggactgagccggtaaatatagagattctcgaagtcactattagcgcctcgttgtcaacgggaatgtcgcttaccacttaaagcataacgccgagaaatcccgtaataaatccagtaaaatacgagcacccgtgccaagttgaatatttgaacccgagtgggtagattccaccgcaaaggacctaaccagatcatttcgcaaacaggaactaaaatcggtagagagcccagacaaaagcctttcctaagagccactccagtggaagcccctactttaggtataaaatgcaatactagtggggctcctaaataaacttctatttttcatggccttctaaaattcactcccaaacccctagctatagaagtctcttatccatcctctaaataaaaatgggagtctattttatttcaccagagttgatcgtaaatttagtctctcaaattttataagttgagggtagaggatgactggagttgctctaaacggacctatcttcaagtgacctcagtgagcccgtttaacggcgtcgacaagtttaatctaacggacaccaaccagagaagagaaccaccgccagcgccgagccaagcgacgttgacatcttggcgcggcacggcatctccctggcgtctggccccctctcgagacttccgctccacctcccaccggtggcggtttccaagtccgttccgcctcctctcacacggcacgaaaccgtgacgggcaccggcagcacggggggattcctttcccaccgctccttccctttcccttcctctcccgccgctataaatagccagccccatccccagcttctttccccaacctcatcttctctcgtgttgttcggcacaacccgatcgatccccaactccctcgtcgtctctcctcgcgagcctcgtcgatcccccgcttcaaggtacggcgatcgattatcttccctctctctaccttctctctcttatagggcctgctagctctgttcctgtttttccatggctgcgaggtacaatagatcggcgatccatggttagggcctgctagttgtgttcctgtttttccatggctgcgaggcacaatagatctgatggcgttatgatggttaacttgtcatactcttgcgatctatggtccctttaggagtttaggacatctatttaatttcggatagttcgagatctgtgatccatggttagtaccctaggcagtggggttagatccgtgctgttatggttcgtagatggattctgattgctcagtaactgggaatcctgggatggttctagctggttcgcagataagatcgatttcatgatatgctatatcttgtttggttgccgtggttccgttaaatctgtctgttatgatcttagtctttgataaggttcggtcgtgctagctacgtcctgtgcagcacttaattgtcaggtcataatttttagcatgccttttttttattggtttggttttgtctgactgggctgtagatagtttcaatctttgtctgactgggctgtagatagtttcaatctacctgtcggtttattttattaaatttggatctgtatgtgtgtcatatatcttcatcttttagatatatcgataggtttatatgttgctgtcggttttttactgttcctttatgagatatattcatgcttagatacatgaaacaacgtgctgttacagtttaatagttcttgtttatctaataaacaaataaggataggtatatgctgcagttagttttactggtactttttttgacatgaacctacggcttaataattagtcttcatcaaataaaaagcatattttttaattatttcgatatacttgaatgatgtcatatgcagcatctgtgtgaatttttggccctgtcttcatatgctgtttatttgtttgggactgtttctttggttgataactcatcctgttgtttggtgatccttttgcaggtgcaaccatgtctccggagaggagaccagttgagattaggccagctacagcagctgatatggccgcggtttgtgatatcgttaaccattacattgagacgtctacagtgaactttaggacagagccacaaacaccacaagagtggattgatgatctagagaggttgcaagatagatacccttggttggttgctgaggttgagggtgttgtggctggtattgcttacgctgggccctggaaggctaggaacgcttacgattggacagttgagagtactgtttacgtgtcacataggcatcaaaggttgggcctaggatccacattgtacacacatttgcttaagtctatggaggcgcaaggttttaagtctgtggttgctgttataggccttccaaacgatccatctgttaggttgcatgaggctttgggatacacagcccggggtacattgcgcgcagctggatacaagcatggtggatggcatgatgttggtttttggcaaagggattttgagttgccagctcctccaaggccagttaggccagttacccagatctgattaattaactaggctactgtagctagctgtgcatgtatgtggtgtggttactaaaataattagtgttttccttttgtttggaagcatatgtgtggtgaataaatgatgaactccgatgttcctctctataaatcttgatgattcgctagctatccgtacgtcgttgttctttgatttgatgatgagattgaaaaatggaatgtcatgctaaggagggtgccgcggcccggccgtgacggccacgagcgaactcctgcaggacaacggagcagcctcctcagcaaatcctaccacctcatttaaatagagtgaggttgatttgctgaggtagcggccgcgttaacaagcttctgcagaattcgtcaacgagatcttgagccaatcaaagaggagtgatgtagacctaaagcaataatggagccatgacgtaagggcttacgcccatacgaaataattaaaggctgatgtgacctgtcggtctctcagaacctttactttttatgtttggcgtgtatttttaaatttccacggcaatgacgatgtgacccaacgagatcttgagccaatcaaagaggagtgatgtagacctaaagcaataatggagccatgacgtaagggcttacgcccatacgaaataattaaaggctgatgtgacctgtcggtctctcagaacctttactttttatatttggcgtgtatttttaaatttccacggcaatgacgatgtgacctgtgcatccgctttgcctataaataagttttagtttgtattgatcgacacggtcgagaagacacggccattctagaaccatcttccacacactcaagccacactattggagaacacacagggacaacacaccataagatccaagggaggcctccgccgccgccggtaaccaccccgcccctctcctctttctttctccgtttttttttccgtctcggtctcgatctttggccttggtagtttgggtgggcgagaggcggcttcgtgcgcgcccagatcggtgcgcgggaggggcgggatctcgcggctggggctctcgccggcgtggatccggcccggatctcgcggggaatggggctctcggatgtagatctgcgatccgccgttgttgggggagatgatggggggtttaaaatttccgccgtgctaaacaagatcaggaagaggggaaaagggcactatggtttatatttttatatatttctgctgcttcgtcaggcttagatgtgctagatctttctttcttctttttgtgggtagaatttgaatccctcagcattgttcatcggtagtttttcttttcatgatttgtgacaaatgcagcctcgtgcggagcttttttgtaggtagaagtgatcaaccatggcccagatcaacaacatggcccagggcatccagaccctgaaccctaactctaacttccacaagccgcaagtgcccaagtctagctccttcctcgtgttcggctccaagaagctcaagaatagcgccaattccatgctggtcctgaagaaagactcgatcttcatgcagaagttctgctcctttcgcatcagtgcttcggttgcgactgcctgcatgctcaccttcgttaggaacgcctggtacgtcgccgctctccctgaggagctgagcgagaagcccttgggtcgcaccatcctagacactccgttagccctttaccgccagcctgacggcgtagtggcggccctgcttgacatctgcccgcataggttcgctccgctcagcgacggcatcctcgtcaacgggcatcttcagtgcccgtaccacgggctggaatttgacggcggtgggcagtgtgtccacaacccgcacggcaacggcgcacggccagcttccctcaacgttaggtcgttccctgttgtcgagcgcgacgcactgatctggatctggcctggcgacccagctctggccgatccaggagccattcccgacttcggttgccgcgtggacccagcctatcggacggtcggcggttacgggcacgtcgattgtaactataagctccttgtggacaaccttatggatttgggccacgctcagtacgtgcaccgggctaacgctcagactgacgcctttgaccgtctcgaaagggaggtcatcgtcggcgacggagagattcaggcgctgatgaagatccctggaggcacgccctctgtgctcatggcgaagtttctcagaggcgcgaacacgcccgtggacgcctggaacgacatccgctggaataaggtctccgcgatgctgaacttcatcgccgttgcgcccgagggcacacccaaagagcagtcaatccacagcagagggacccatattcttacaccggaaaccgaggctagttgccactacttcttcggctcgtcacggaatttcgggatagacgatccggagatggacggtgttcttcgatcttggcaagcgcaagctctcgtcaaggaagataaggtggtcgtggaggctatcgagcgtaggcgcgcctacgttgaggcgaacggtattaggcccgcgatgctgtcctgcgacgaggccgcagttagagtgtcgcgcgagatagaaaagctggagcagctagaggccgcctgaggtaccgagctcgtcaatcactagtgaattctgcatgcgtttggacgtatgctcattcaggttggagccaatttggttgatgtgtgtgcgagttcttgcgagtctgatgagacatctctgtattgtgtttctttccccagtgttttctgtacttgtgtaatcggctaatcgccaacagattcggcgatgaataaatgagaaataaattgttctgattttgagtgcaaaaaaaaaggaattagatctgtgtgtgttttttggatccccggggcggccgcacaacaaacgaatacgtcctgcttggcctactaggccaacgcaggcgctggccgtgacggccacgagcgaactgatatcgaattctagggataacagggtaatccacgtgtagctaaacgcgccctcatctaagcccccatttggacgtgaatgtagacacgtcgaaataaagatttccgaattagaataatttgtttattgctttcgcctataaatacgacggatcgtaatttgtcgttttatcaaaatgtactttcattttataataacgctgcggacatctacatttttgaattgaaaaaaaattggtaattactctttctttttctccata

SEQ ID NO: 10 - DNA, 9259 bp, Artificial Sequence
  Recombinant
gttgatattttgacccaaagacatgccattctcattgttttcagttttatcctaccaatgtagtaacccaaacagtttaattacaagtgaatcaactggaaacaagatctacagactgcacacagcacattaacaattctgcgccaaatgaatgacagagtgatttataggcactaagctggttttcatcatgaattttgatcagagcataaaccttgttgacaacagaatagaatcaaacaagctgctcagctcagatggaccaaaataatgaacgcgcgcacagtatattgaaccaaaatagtgaacgcacagtagaaaacagacggagaagctagtgcacactaaaaatagaactcactgatgcatttttaaccgaatcattaaaaaacagaccaacatgattagaccagctatcaaaagacacactgctgagaatcaacaactgctatatgtgtgatctacctgaaataaacagatgcagttttttgtccctacagaccaacatgttttaatcagaatgccaatgataaatccttagagatctggagagcaaactaattaaccactgagaatcaacaactgctataatccttagagatctggagagcacactaattaaccactgagcctctttggtcagcatgcagaaatccccaaaactatactgtaattcgaaacccataagcgcacatcaaagcaactccattgttgatggttgggaatgttaaaaatatggttgtggacaccaattgccgtaaacaaacccacagggagaacatgagtatgaacaatcaaaactaacatgaataagtggatgttcagattaagtaaggaaaatggtgcacagattaagaacagagcaatgtatagcacaagtggaaattacaaaccttttttcacaaaattacaatctctagacagcacacagcaagatcttggaatggatgagggtgatgaatcggtgaaaaaagacagcacacagcaagatctctagaacagaacatgaaatgttggagagtggggatgggttgtagacctaacctctgtccatccttttaatagccgtcgctgccaggtatggaatagggcgccgtgagtgccgtcgagggcgcgcgcaggggcgcggtttggtgtgggcgggatacccggcgcggtcgggaaaccccacggcggtcatcacggcgagccgggggaggggggggttggcggggtggcaggcggtcgctgccaggtattgatgtgcgccagtcagcatcatcacaccaaaagttaggcccgaatagtttgaaattagaaagctcgcaattgaggtctgtcgaggaggttaacctaggtactgaattaccctgttatccctaactagatatcgaattctaactataacggtcctaaggtagcgaatcgttcttcttggcgcgccaagacgcaaactcggaccggttcaagccgtcaaggcacttctatgcaaccacagtcaacttgaatgccgcttgagtgccttctcaagtttttttttcttgcaaaaatcatttcttttttttaaaaaaagtataatttggatcgtgcaaatttctctctaggtgtgtgtgtgactgtgtgagtaacaatttctctagttgtgcgcgactgctgcttactttggagattacaatatctttctaaaatgcttcgattacttatttataaaccgtctctaaggccaattgctcaagattcattcaacaattgaaacgtctcacatgattaaatcatataaagtttctaagtcttgtttgacaagatttttttagattttcatctaaattggatgaaactatcaaacactaattttaaaaaatataagagaagctccggagataaaaggtcgtctatgttattataagagtaaagtcgtctattctcttcgtcccaacatatataattctaagcatgaattgctttctttttggacaaaaggagcatgccacaacacaagaatgatgtcaccgtcatgcttggatccttttatggtaaagcttcaccttctataatctaacaatagagaaatcagggaaaaatcatgttttggttgtttttatttctaacctccacaataactttggtttaccattttttgtttgattttagttttagagaagcgtttataacaggacctaaaatcttttttcagtacacagtacaacgcagacgctcatacacgcacgcacactcacctctatgaacacacgtaagaaaaccctacaccttgagcaccttcgaaggactgagccggtaaatatagagattctcgaagtcactattagcgcctcgttgtcaacgggaatgtcgcttaccacttaaagcataacgccgagaaatcccgtaataaatccagtaaaatacgagcacccgtgccaagttgaatatttgaacccgagtgggtagattccaccgcaaaggacctaaccagatcatttcgcaaacaggaactaaaatcggtagagagcccagacaaaagcctttcctaagagccactccagtggaagcccctactttaggtataaaatgcaatactagtggggctcctaaataaacttctatttttcatggccttctaaaattcactcccaaacccctagctatagaagtctcttatccatcctctaaataaaaatgggagtctattttatttcaccagagttgatcgtaaatttagtctctcaaattttataagttgagggtagaggatgactggagttgctctaaacggacctatcttcaagtgacctcagtgagcccgtttaacggcgtcgacaagtttaatctaacggacaccaaccagagaagagaaccaccgccagcgccgagccaagcgacgttgacatcttggcgcggcacggcatctccctggcgtctggccccctctcgagacttccgctccacctcccaccggtggcggtttccaagtccgttccgcctcctctcacacggcacgaaaccgtgacgggcaccggcagcacggggggattcctttcccaccgctccttccctttcccttcctctcccgccgctataaatagccagccccatccccagcttctttccccaacctcatcttctctcgtgttgttcggcacaacccgatcgatccccaactccctcgtcgtctctcctcgcgagcctcgtcgatcccccgcttcaaggtacggcgatcgattatcttccctctctctaccttctctctcttatagggcctgctagctctgttcctgtttttccatggctgcgaggtacaatagatcggcgatccatggttagggcctgctagttgtgttcctgtttttccatggctgcgaggcacaatagatctgatggcgttatgatggttaacttgtcatactcttgcgatctatggtccctttaggagtttaggacatctatttaatttcggatagttcgagatctgtgatccatggttagtaccctaggcagtggggttagatccgtgctgttatggttcgtagatggattctgattgctcagtaactgggaatcctgggatggttctagctggttcgcagataagatcgatttcatgatatgctatatcttgtttggttgccgtggttccgttaaatctgtctgttatgatcttagtctttgataaggttcggtcgtgctagctacgtcctgtgcagcacttaattgtcaggtcataatttttagcatgccttttttttattggtttggttttgtctgactgggctgtagatagtttcaatctttgtctgactgggctgtagatagtttcaatctacctgtcggtttattttattaaatttggatctgtatgtgtgtcatatatcttcatcttttagatatatcgataggtttatatgttgctgtcggttttttactgttcctttatgagatatattcatgcttagatacatgaaacaacgtgctgttacagtttaatagttcttgtttatctaataaacaaataaggataggtatatgctgcagttagttttactggtactttttttgacatgaacctacggcttaataattagtcttcatcaaataaaaagcatattttttaattatttcgatatacttgaatgatgtcatatgcagcatctgtgtgaatttttggccctgtcttcatatgctgtttatttgtttgggactgtttctttggttgataactcatcctgttgtttggtgatccttttgcaggtgcaaccatgtctccggagaggagaccagttgagattaggccagctacagcagctgatatggccgcggtttgtgatatcgttaaccattacattgagacgtctacagtgaactttaggacagagccacaaacaccacaagagtggattgatgatctagagaggttgcaagatagatacccttggttggttgctgaggttgagggtgttgtggctggtattgcttacgctgggccctggaaggctaggaacgcttacgattggacagttgagagtactgtttacgtgtcacataggcatcaaaggttgggcctaggatccacattgtacacacatttgcttaagtctatggaggcgcaaggttttaagtctgtggttgctgttataggccttccaaacgatccatctgttaggttgcatgaggctttgggatacacagcccggggtacattgcgcgcagctggatacaagcatggtggatggcatgatgttggtttttggcaaagggattttgagttgccagctcctccaaggccagttaggccagttacccagatctgattaattaactaggctactgtagctagctgtgcatgtatgtggtgtggttactaaaataattagtgttttccttttgtttggaagcatatgtgtggtgaataaatgatgaactccgatgttcctctctataaatcttgatgattcgctagctatccgtacgtcgttgttctttgatttgatgatgagattgaaaaatggaatgtcatgctaaggagggtgccgcggcccggccgtgacggccacgagcgaactcctgcaggacaacggagcagcctcctcagcaaatcctaccacctcatttaaatagagtgaggttgatttgctgaggtagcggccgcgttaacaagcttctgcagaattcgtcaacgagatcttgagccaatcaaagaggagtgatgtagacctaaagcaataatggagccatgacgtaagggcttacgcccatacgaaataattaaaggctgatgtgacctgtcggtctctcagaacctttactttttatgtttggcgtgtatttttaaatttccacggcaatgacgatgtgacccaacgagatcttgagccaatcaaagaggagtgatgtagacctaaagcaataatggagccatgacgtaagggcttacgcccatacgaaataattaaaggctgatgtgacctgtcggtctctcagaacctttactttttatatttggcgtgtatttttaaatttccacggcaatgacgatgtgacctgtgcatccgctttgcctataaataagttttagtttgtattgatcgacacggtcgagaagacacggccattctagaaccatcttccacacactcaagccacactattggagaacacacagggacaacacaccataagatccaagggaggcctccgccgccgccggtaaccaccccgcccctctcctctttctttctccgtttttttttccgtctcggtctcgatctttggccttggtagtttgggtgggcgagaggcggcttcgtgcgcgcccagatcggtgcgcgggaggggcgggatctcgcggctggggctctcgccggcgtggatccggcccggatctcgcggggaatggggctctcggatgtagatctgcgatccgccgttgttgggggagatgatggggggtttaaaatttccgccgtgctaaacaagatcaggaagaggggaaaagggcactatggtttatatttttatatatttctgctgcttcgtcaggcttagatgtgctagatctttctttcttctttttgtgggtagaatttgaatccctcagcattgttcatcggtagtttttcttttcatgatttgtgacaaatgcagcctcgtgcggagcttttttgtaggtagaagtgatcaaccatggcccagatcaacaacatggcccagggcatccagaccctgaaccctaactctaacttccacaagccgcaagtgcccaagtctagctccttcctcgtgttcggctccaagaagctcaagaatagcgccaattccatgctggtcctgaagaaagactcgatcttcatgcagaagttctgctcctttcgcatcagtgcttcggttgcgactgcctgcatgctcaccttcgttaggaacgcctggtacgtcgccgctctccctgaggagctgagcgagaagcccttgggtcgcaccatcctagacactccgttagccctttaccgccagcctgacggcgtagtggcggccctgcttgacatctgcccgcataggttcgctccgctcagcgacggcatcctcgtcaacgggcatcttcagtgcccgtaccacgggctggaatttgacggcggtgggcagtgtgtccacaacccgcacggcaacggcgcacggccagcttccctcaacgttaggtcgttccctgttgtcgagcgcgacgcactgatctggatctggcctggcgacccagctctggccgatccaggagccattcccgacttcggttgccgcgtggacccagcctatcggacggtcggcggttacgggcacgtcgattgtaactataagctccttgtggacaaccttatggatttgggccacgctcagtacgtgcaccgggctaacgctcagactgacgcctttgaccgtctcgaaagggaggtcatcgtcggcgacggagagattcaggcgctgatgaagatccctggaggcacgccctctgtgctcatggcgaagtttctcagaggcgcgaacacgcccgtggacgcctggaacgacatccgctggaataaggtctccgcgatgctgaacttcatcgccgttgcgcccgagggcacacccaaagagcagtcaatccacagcagagggacccatattcttacaccggaaaccgaggctagttgccactacttcttcggctcgtcacggaatttcgggatagacgatccggagatggacggtgttcttcgatcttggcaagcgcaagctctcgtcaaggaagataaggtggtcgtggaggctatcgagcgtaggcgcgcctacgttgaggcgaacggtattaggcccgcgatgctgtcctgcgacgaggccgcagttagagtgtcgcgcgagatagaaaagctggagcagctagaggccgcctgaggtaccgagctcgtcaatcactagtgaattctgcatgcgtttggacgtatgctcattcaggttggagccaatttggttgatgtgtgtgcgagttcttgcgagtctgatgagacatctctgtattgtgtttctttccccagtgttttctgtacttgtgtaatcggctaatcgccaacagattcggcgatgaataaatgagaaataaattgttctgattttgagtgcaaaaaaaaaggaattagatctgtgtgtgttttttggatccccggggcggccgcacaacaaacgaatacgtcctgcttggcctactaggccaacgcaggcgctggccgtgacggccacgagcgaactgatatcgaattctagggataacagggtaatccacgtgtagctaaacgcgccctcatctaagcccccatttggacgtgaatgtagacacgtcgaaataaagatttccgaattagaataatttgtttattgctttcgcctataaatacgacggatcgtaatttgtcgttttatcaaaatgtactttcattttataataacgctgcggacatctacatttttgaattgaaaaaaaattggtaattactctttctttttctccatagcattcgcaatacagttagatgcgagtgaagcacgataagtcacaaccataatacatactattagaatccggctctttgccgagtgctttttttgggcactcggcaaagacttctttaccggcaaagtcctactctcggtaacgaccacgtttaccgagagcaggacgctcggtacagggagacactcggcaaagacctctttgtcgagtgccaaacgctcggcaaagggccgtcagcagccgtctatagcagatgtttattatctttgccgagcgccaagcgttggcactcggcaaaacaagtgttgccgagtgcttaaattggacactcggcaaaatatatttttcttttttctttttgcaaccaaactttctgtggtttgttcctacactatgtagacatacatgttccattttggcacaattataaaagtgtttgctataaatattagattttgttcgtttaattgaattttctcggataattcagatttgaactacaagtcactcaaaaaatggaaaaccatgaatgcaaaaatgatatccatgttatttagcacaagttacggccgatttcaggagtagacccgaatttttgagcaccatgctcacgaaacatgactgtgaacttgtcatccagttgttttaaaattgtataaaacacaaacaaaatcaaaaaatcatgaaacttgtccacatgtcatgatatcatcatatgtagaggttgtgataaaaagttgaaaatatttcgtgaaagttgtccatagttcactgagcctctttgtcgagtgtcacactcggcaaagcctttgtcgagtgcttcagacactcggcaaataagttgtttccagtagtgacattaatagaaaaagagtgcatagttcgttcacatagctaactaattggttcattacaaagaaacattagaacaagcataatgatgacttggacataatgaaataaaatacataggttgagggaaccaaacataatggaacacagaacaaatagaggacaacatcatagaaaacgacataacttcacatgggttttacgccaattgctccacgccaagtccataagtgctcgatgagatcatgttgaagttggttgtatcatttgagactagtgatgttgtggtgggagcatagccactctgtacgaacttcagggattgtgatgagagatccacgtgcactccaattgcggcaaactcaacattacttgcacgtgggaccttgtcctcgacaa

SEQ ID NO: 11 - DNA, 33 bp, Artificial Sequence
  Recombinant
gaattgaaaaaaaattggtaattactctttctt

SEQ ID NO: 12 - DNA, 24 bp, Artificial Sequence
  Recombinant
atcgtgcttcactcgcatctaact

SEQ ID NO: 13 - DNA, 19 bp, Artificial Sequence
  Recombinant
ctccatagcattcgcaata

SEQ ID NO: 14 - DNA, 81 bp, Artificial Sequence
  Recombinant
attagaaagctcgcaattgaggtctgtcgaggaggttaacctaggtactgaattaccctgttatccctaactagatatcga

SEQ ID NO: 15 - DNA, 61 bp, Artificial Sequence
  Recombinant
tggcgcgccaagacgcaaactcggaccggttcaagccgtcaaggcacttctatgcaaccac

SEQ ID NO: 16 - DNA, 59 bp, Artificial Sequence
  Recombinant
atcctgttgtttggtgatccttttgcaggtgcaaccatgtctccggagaggagaccagt

SEQ ID NO: 17 - DNA, 56 bp, Artificial Sequence
  Recombinant
ccagttaggccagttacccagatctgattaattaactaggctactgtagctagctg

SEQ ID NO: 18 - DNA, 99 bp, Artificial Sequence
  Recombinant
aaaaatggaatgtcatgctaaggagggtgccgcggcccggccgtgacggccacgagcgaactcctgcaggacaacggagcagcctcctcagcaaatcct

SEQ ID NO: 19 - DNA, 56 bp, Artificial Sequence
  Recombinant
tgaggttgatttgctgaggtagcggccgcgttaacaagcttctgcagaattcgtca

SEQ ID NO: 20 - DNA, 55 bp, Artificial Sequence
  Recombinant
aggtagaagtgatcaaccatggcccagatcaacaacatggcccagggcatccaga

SEQ ID NO: 21 - DNA, 91 bp, Artificial Sequence
  Recombinant
cgcgagatagaaaagctggagcagctagaggccgcctgaggtaccgagctcgtcaatcactagtgaattctgcatgcgtttggacgtatgc

SEQ ID NO: 22 - DNA, 67 bp, Artificial Sequence
  Recombinant
ctagggataacagggtaatccacgtgtagctaaacgcgccctcatctaagcccccatttggacgtga